European Patent Specification EP 3 313 883 B1, published December 6, 2023. Title: PD-1 Immune Modulating Agents. Applicant: Memorial Sloan-Kettering Cancer Center Eureka Therapeutics, Inc. Brentjens, Renier J Jackson, Hollie J Liu, Cheng. The sequence listing filed with the application follows.

SEQUENCE LISTING (143 sequences)

SEQ ID NO: 1 - protein, 6 aa, Artificial Sequence
  Homo sapiens
QSISSY

SEQ ID NO: 2 - protein, 9 aa, Homo sapiens
QQSYSTPLT

SEQ ID NO: 3 - protein, 8 aa, Homo sapiens
GFTSSSYW

SEQ ID NO: 4 - protein, 8 aa, Homo sapiens
IKQDGSEK

SEQ ID NO: 5 - protein, 9 aa, Homo sapiens
ARGGWSYDM

SEQ ID NO: 6 - protein, 110 aa, Homo sapiens
DIQMTQSPSSLSASVGDRVTITCRASQSISSYLNWYQQKPGKAPKLLIYAASSLQSGVPSRFSGSGSGTDFTLTISSLQPEDFATYYCQQSYSTPLTFGGGTKVEIKRSR

SEQ ID NO: 7 - DNA, 324 bp, Homo sapiens
gacatccagatgacccagtctccatcctccctgtctgcatctgtaggagacagagtcaccatcacttgccgggcaagtcagagcattagcagctatttaaattggtatcagcagaaaccagggaaagcccctaagctcctgatctatgctgcatccagtttgcaaagtggggtcccatcaaggttcagtggcagtggatctgggacagatttcactctcaccatcagcagtctgcaacctgaagattttgcaacttactactgtcaacagagttacagtaccccgctcactttcggcggagggaccaaggtggagatcaaacgt

SEQ ID NO: 8 - protein, 116 aa, Homo sapiens
EVQLVESGGGLVQPGGSLRLSCAASGFTSSSYWMSWVRQAPGRGLEWVANIKQDGSEKYYVDSVKGRFTISRDNAKNSLYLQMNSLRAEDTAVYYCARGGWSYDMWGQGTLVTVSS

SEQ ID NO: 9 - DNA, 348 bp, Homo sapiens
gaggtgcagctggtggagtctgggggaggcttggtccagcctggggggtccctgagactctcctgtgcagcctctggattcacctctagtagctattggatgagctgggtccgccaggctccagggagagggctggagtgggtggccaacataaagcaagatggaagtgagaagtactatgtggactctgtgaagggccgattcaccatctccagagacaacgccaagaactcactgtatctgcaaatgaacagcctgagagccgaggacactgccgtgtattactgtgcgcgcggtggttggtcttacgatatgtggggtcaaggtactctggtgaccgtctcctca

SEQ ID NO: 10 - protein, 259 aa, Homo sapiens
DIQMTQSPSSLSASVGDRVTITCRASQSISSYLNWYQQKPGKAPKLLIYAASSLQSGVPSRFSGSGSGTDFTLTISSLQPEDFATYYCQQSYSTPLTFGGGTKVEIKRSRGGGGSGGGGSGGGGSEVQLVESGGGLVQPGGSLRLSCAASGFTSSSYWMSWVRQAPGRGLEWVANIKQDGSEKYYVDSVKGRFTISRDNAKNSLYLQMNSLRAEDTAVYYCARGGWSYDMWGQGTLVTVSSHHHHHHGAYPYDVPDYAS

SEQ ID NO: 11 - DNA, 717 bp, Homo sapiens
gacatccagatgacccagtctccatcctccctgtctgcatctgtaggagacagagtcaccatcacttgccgggcaagtcagagcattagcagctatttaaattggtatcagcagaaaccagggaaagcccctaagctcctgatctatgctgcatccagtttgcaaagtggggtcccatcaaggttcagtggcagtggatctgggacagatttcactctcaccatcagcagtctgcaacctgaagattttgcaacttactactgtcaacagagttacagtaccccgctcactttcggcggagggaccaaggtggagatcaaacgtggtggtggtggtagcggcggcggcggctctggtggtggtggatccgaggtgcagctggtggagtctgggggaggcttggtccagcctggggggtccctgagactctcctgtgcagcctctggattcacctctagtagctattggatgagctgggtccgccaggctccagggagagggctggagtgggtggccaacataaagcaagatggaagtgagaagtactatgtggactctgtgaagggccgattcaccatctccagagacaacgccaagaactcactgtatctgcaaatgaacagcctgagagccgaggacactgccgtgtattactgtgcgcgcggtggttggtcttacgatatgtggggtcaaggtactctggtgaccgtctcctca

SEQ ID NO: 12 - protein, 9 aa, Homo sapiens
SSNIGAGYA

SEQ ID NO: 13 - protein, 11 aa, Homo sapiens
QSYDSSLSGVI

SEQ ID NO: 14 - protein, 8 aa, Homo sapiens
GYTLTELS

SEQ ID NO: 15 - protein, 8 aa, Homo sapiens
FDPEDGET

SEQ ID NO: 16 - protein, 9 aa, Homo sapiens
ARAYYGFDQ

SEQ ID NO: 17 - protein, 112 aa, Homo sapiens
QSVLTQPPSVSGAPGQRVTISCTGSSSNIGAGYAVNWYQLLPGTAPKLLISTNNNRPSGVPDRFSGSQFGASASLAITGLQAEDEADYYCQSYDSSLSGVIFGGGTKLTVLG

SEQ ID NO: 18 - DNA, 336 bp, Homo sapiens
cagtctgtgttgacgcagccgccctcagtgtctggggccccagggcagagggtcaccatctcctgcactgggagcagctccaacatcggggcaggttatgctgtaaattggtaccagcttcttccaggaacagcccccaaactcctcatctctactaacaacaatcggccctcaggggtccctgaccgattctctggctcccagtttggcgcctctgcctccctggccatcactggactccaggctgaggatgaggctgattattactgccagtcctatgacagtagtctgagtggtgtgatattcggcggagggaccaagctgaccgtcctaggt

SEQ ID NO: 19 - protein, 116 aa, Homo sapiens
EVQLVQSGAEVKKPGASVKVSCKVSGYTLTELSMHWVRQAPGKGLEWMGGFDPEDGETIYAQKFQGRVTMTEDTSTDTAYMELSSLRSEDTAVYYCARAYYGFDQWGQGTLVTVSS

SEQ ID NO: 20 - DNA, 348 bp, Homo sapiens
gaagtgcagctggtgcagtctggggctgaggtgaagaagcctggggcctcagtgaaggtctcctgcaaggtttccggatacaccctcactgaattatccatgcactgggtgcgacaggctcctggaaaagggcttgagtggatgggaggttttgatcctgaagatggtgaaacaatctacgcacagaagttccagggcagagtcaccatgaccgaggacacatctacagacacagcctacatggagctgagcagcctgaggtctgaggacactgccgtgtattactgtgcgcgcgcttactacggtttcgatcagtggggtcaaggtactctggtgaccgtctcctca

SEQ ID NO: 21 - protein, 257 aa, Homo sapiens
DIQMTQSPSSLSASVGDRVTITCRASQSISSYLNWYQQKPGKAPKLLIYAASSLQSGVPSRFSGSGSGTDFTLTISSLQPEDFATYYCQQSYSTPLTFGGGTKVEIKRGGGGSGGGGSGGGGSEVQLVQSGAEVKKPGASVKVSCKVSGYTLTELSMHWVRQAPGKGLEWMGGFDPEDGETIYAQKFQGRVTMTEDTSTDTAYMELSSLRSEDTAVYYCARAYYGFDQWGQGTLVTVSSHHHHHHGAYPYDVPDYAS

SEQ ID NO: 22 - protein, 729 aa, Homo sapiens
CAGTCTGTGTTGACGCAGCCGCCCTCAGTGTCTGGGGCCCCAGGGCAGAGGGTCACCATCTCCTGCACTGGGAGCAGCTCCAACATCGGGGCAGGTTATGCTGTAAATTGGTACCAGCTTCTTCCAGGAACAGCCCCCAAACTCCTCATCTCTACTAACAACAATCGGCCCTCAGGGGTCCCTGACCGATTCTCTGGCTCCCAGTTTGGCGCCTCTGCCTCCCTGGCCATCACTGGACTCCAGGCTGAGGATGAGGCTGATTATTACTGCCAGTCCTATGACAGTAGTCTGAGTGGTGTGATATTCGGCGGAGGGACCAAGCTGACCGTCCTAGGTGGTGGTGGTGGTAGCGGCGGCGGCGGCTCTGGTGGTGGTGGATCCGAAGTGCAGCTGGTGCAGTCTGGGGCTGAGGTGAAGAAGCCTGGGGCCTCAGTGAAGGTCTCCTGCAAGGTTTCCGGATACACCCTCACTGAATTATCCATGCACTGGGTGCGACAGGCTCCTGGAAAAGGGCTTGAGTGGATGGGAGGTTTTGATCCTGAAGATGGTGAAACAATCTACGCACAGAAGTTCCAGGGCAGAGTCACCATGACCGAGGACACATCTACAGACACAGCCTACATGGAGCTGAGCAGCCTGAGGTCTGAGGACACTGCCGTGTATTACTGTGCGCGCGCTTACTACGGTTTCGATCAGTGGGGTCAAGGTACTCTGGTGACCGTCTCCTCA

SEQ ID NO: 23 - protein, 8 aa, Homo sapiens
SSNIGNNA

SEQ ID NO: 24 - protein, 11 aa, Homo sapiens
AAWDDSVNGYV

SEQ ID NO: 25 - protein, 8 aa, Homo sapiens
GYTFTRFG

SEQ ID NO: 26 - protein, 8 aa, Homo sapiens
ISVNNGNT

SEQ ID NO: 27 - protein, 10 aa, Homo sapiens
ARYMYGRRDS

SEQ ID NO: 28 - protein, 111 aa, Homo sapiens
QAVLTQPPSMSEAPRQRVTISCSGSSSNIGNNAVNWYQQLPGKAPKLLIYYNDLLSSGVSDRFSGSKSGTSASLAISGLQSEDEADYYCAAWDDSVNGYVFGTGTKVTVLG

SEQ ID NO: 29 - DNA, 333 bp, Homo sapiens
caggctgtgctgactcagccaccctcgatgtctgaagcccccaggcagagggtcaccatctcctgttctggaagcagctccaacatcggaaataatgctgtaaactggtaccagcagctcccaggaaaggctcccaaactcctcatctattataatgatctgctgtcctcaggggtctctgaccgattctctggctccaagtctggcacctcagcctccctggccatcagtgggctccagtctgaggatgaggctgattattactgtgcagcatgggatgacagtgtgaatggttatgtcttcggaactgggaccaaggtcaccgtcctaggt

SEQ ID NO: 30 - protein, 117 aa, Homo sapiens
EVQLVQSGAEVKKPGDSVKVSCKASGYTFTRFGFSWVRQAPGQGLEWMGWISVNNGNTKYAQKYQGRVTMTTDTSTSTAYMELRSLRSDDTAVYYCARYMYGRRDSWGQGTLVTVSS

SEQ ID NO: 31 - DNA, 351 bp, Homo sapiens
gaggtccagctggtgcagtctggagctgaggtgaagaagcctggggactcagtgaaggtctcctgcaaggcttctggttacacctttaccagatttggtttcagctgggtgcgacaggcccctggacaagggcttgagtggatgggatggatcagcgttaataatggtaacacaaagtatgcacagaagtaccagggcagagtcaccatgaccacagacacatccacgagcacagcctacatggagctgaggagcctgaggtctgacgacactgccgtgtattactgtgcgcgctacatgtacggtcgtcgtgattcttggggtcaaggtactctggtgaccgtctcctca

SEQ ID NO: 32 - protein, 266 aa, Homo sapiens
QAVLTQPPSMSEAPRQRVTISCSGSSSNIGNNAVNWYQQLPGKAPKLLIYYNDLLSSGVSDRFSGSKSGTSASLAISGLQSEDEADYYCAAWDDSVNGYVFGTGTKVTVLGGSRGGGGSGGGGSGGGGSEVQLVQSGAEVKKPGDSVKVSCKASGYTFTRFGFSWVRQAPGQGLEWMGWISVNNGNTKYAQKYQGRVTMTTDTSTSTAYMELRSLRSDDTAVYYCARYMYGRRDSWGQGTLVTVSSGQHHHHHHGAYPYDVPDYAS

SEQ ID NO: 33 - DNA, 804 bp, Homo sapiens
caggctgtgctgactcagccaccctcgatgtctgaagcccccaggcagagggtcaccatctcctgttctggaagcagctccaacatcggaaataatgctgtaaactggtaccagcagctcccaggaaaggctcccaaactcctcatctattataatgatctgctgtcctcaggggtctctgaccgattctctggctccaagtctggcacctcagcctccctggccatcagtgggctccagtctgaggatgaggctgattattactgtgcagcatgggatgacagtgtgaatggttatgtcttcggaactgggaccaaggtcaccgtcctaggtggttctagaggtggtggtggtagcggcggcggcggctctggtggtggtggatccgaggtccagctggtgcagtctggagctgaggtgaagaagcctggggactcagtgaaggtctcctgcaaggcttctggttacacctttaccagatttggtttcagctgggtgcgacaggcccctggacaagggcttgagtggatgggatggatcagcgttaataatggtaacacaaagtatgcacagaagtaccagggcagagtcaccatgaccacagacacatccacgagcacagcctacatggagctgaggagcctgaggtctgacgacactgccgtgtattactgtgcgcgctacatgtacggtcgtcgtgattcttggggtcaaggtactctggtgaccgtctcctcagccggccagcaccatcaccatcaccatggcgcatacccgtacgacgttccggactacgcttcttag

SEQ ID NO: 34 - protein, 6 aa, Homo sapiens
NIGSKS

SEQ ID NO: 35 - protein, 10 aa, Homo sapiens
QVWDNHSDVV

SEQ ID NO: 36 - protein, 8 aa, Homo sapiens
RNKFSSYA

SEQ ID NO: 37 - protein, 8 aa, Homo sapiens
ISGSGGTT

SEQ ID NO: 38 - protein, 10 aa, Homo sapiens
ARWYSSYYDV

SEQ ID NO: 39 - protein, 108 aa, Homo sapiens
QSVLTQPPSVSVAPGKTARITCGGNNIGSKSVHWYQQKPGQAPVLVIYYDSDRPSGIPERFSGSNSGNTATLTISRVEAGDEADYYCQVWDNHSDVVFGGGTKLTVLG

SEQ ID NO: 40 - DNA, 324 bp, Homo sapiens
cagtctgtgctgactcagccaccctcagtgtcagtggccccaggaaagacggccaggattacctgtgggggaaacaacattggaagtaaaagtgtgcactggtaccagcagaagccaggccaggcccctgtgctggtcatctattatgatagcgaccggccctcagggatccctgagcgattctctggctccaactctgggaacacggccaccctgaccatcagcagggtcgaagccggggatgaggccgactattactgtcaggtctgggataatcatagtgatgtggtattcggcggagggaccaagctgaccgtcctaggt

SEQ ID NO: 41 - protein, 120 aa, Homo sapiens
QVQLVESGGGLVQPGGSLRLSCAASGYTRNKFSSYAMSWVRQAPGKGLEWVSGISGSGGTTYYADSVKGRFTISRDNSKNTQYLQLDSLRAEDTAVYYCARWYSSYYDVWGQGTLVTVSS

SEQ ID NO: 42 - DNA, 360 bp, Homo sapiens
caggtgcagctggtggagtctgggggaggcttggtacagcctggggggtccctgagactctcctgtgcagcctctggatacacccgtaacaaatttagcagctatgccatgagctgggtccgccaggctccagggaagggcctggaatgggtctcaggtattagtggtagtggtggtactacatactatgcagactccgtgaagggccggttcaccatctccagagacaattccaagaacacgcagtatctgcaattggacagcctgagagccgaggacacggccgtatattactgtgcgcgctggtactcttcttactacgatgtttggggtcaaggtactctggtgaccgtctcctca

SEQ ID NO: 43 - protein, 261 aa, Homo sapiens
QSVLTQPPSVSVAPGKTARITCGGNNIGSKSVHWYQQKPGQAPVLVIYYDSDRPSGIPERFSGSNSGNTATLTISRVEAGDEADYYCQVWDNHSDVVFGGGTKLTVLGGGGGSGGGGSGGGGSQVQLVESGGGLVQPGGSLRLSCAASGYTRNKFSSYAMSWVRQAPGKGLEWVSGISGSGGTTYYADSVKGRFTISRDNSKNTQYLQLDSLRAEDTAVYYCARWYSSYYDVWGQGTLVTVSSHHHHHHGAYPYDVPDYAS

SEQ ID NO: 44 - DNA, 786 bp, Homo sapiens
cagtctgtgctgactcagccaccctcagtgtcagtggccccaggaaagacggccaggattacctgtgggggaaacaacattggaagtaaaagtgtgcactggtaccagcagaagccaggccaggcccctgtgctggtcatctattatgatagcgaccggccctcagggatccctgagcgattctctggctccaactctgggaacacggccaccctgaccatcagcagggtcgaagccggggatgaggccgactattactgtcaggtctgggataatcatagtgatgtggtattcggcggagggaccaagctgaccgtcctaggtggtggtggtggtagcggcggcggcggctctggtggtggtggatcccaggtgcagctggtggagtctgggggaggcttggtacagcctggggggtccctgagactctcctgtgcagcctctggatacacccgtaacaaatttagcagctatgccatgagctgggtccgccaggctccagggaagggcctggaatgggtctcaggtattagtggtagtggtggtactacatactatgcagactccgtgaagggccggttcaccatctccagagacaattccaagaacacgcagtatctgcaattggacagcctgagagccgaggacacggccgtatattactgtgcgcgctggtactcttcttactacgatgtttggggtcaaggtactctggtgaccgtctcctcacaccatcaccatcaccatggcgcatacccgtacgacgttccggactacgcttcttag

SEQ ID NO: 45 - protein, 10 aa, Homo sapiens
QVWDSSSDYV

SEQ ID NO: 46 - protein, 8 aa, Homo sapiens
GFTFSSYA

SEQ ID NO: 47 - protein, 8 aa, Homo sapiens
ISGSGGST

SEQ ID NO: 48 - protein, 10 aa, Homo sapiens
ARNYISMFDS

SEQ ID NO: 49 - protein, 108 aa, Homo sapiens
QSVLTQPPSVSVAPGKTARITCGGNNIGSKSVHWYQQRPGQAPVLVIYYDSDRPSGIPERFSGSNSGNTATLTISRVEAGDEADYYCQVWDSSSDYVFGIGTKVTVLG

SEQ ID NO: 50 - DNA, 324 bp, Homo sapiens
cagtctgtgctgactcagccaccctcagtgtcagtggccccaggaaagacggccaggattacctgtgggggaaacaacattggaagtaaaagtgtgcactggtaccagcagaggccaggccaggcccctgtgctggtcatctattatgatagcgaccggccctcagggatccctgagcgattctctggctccaactctgggaacacggccaccctgaccatcagcagggtcgaagccggggatgaggccgactattactgtcaggtgtgggatagtagtagtgattatgtcttcggaattgggaccaaggtcaccgtcctaggt

SEQ ID NO: 51 - protein, 117 aa, Homo sapiens
EVQLVESGGGLIQPGGSLRLSCAASGFTFSSYAMSWVRQAPGKGLEWVSAISGSGGSTYYADSVKGRFTISRDNSKNTLYLQMNSLRAEDTAVYYCARNYISMFDSWGQGTLVTVSS

SEQ ID NO: 52 - DNA, 351 bp, Homo sapiens
gaggtgcagctggtggagtctggaggaggcttgatccagcctggggggtccctgagactctcctgtgcagcctctggattcacctttagcagctatgccatgagctgggtccgccaggctccagggaaggggctggagtgggtctcagctattagtggtagtggtggtagcacatactacgcagactccgtgaagggccggttcaccatctccagagacaattccaagaacacgctgtatctgcaaatgaacagcctgagagccgaggacacggccgtatattactgtgcgcgcaactacatctctatgttcgattcttggggtcaaggtactctggtgaccgtctcctca

SEQ ID NO: 53 - protein, 258 aa, Homo sapiens
QSVLTQPPSVSVAPGKTARITCGGNNIGSKSVHWYQQRPGQAPVLVIYYDSDRPSGIPERFSGSNSGNTATLTISRVEAGDEADYYCQVWDSSSDYVFGIGTKVTVLGGGGGSGGGGSGGGGSEVQLVESGGGLIQPGGSLRLSCAASGFTFSSYAMSWVRQAPGKGLEWVSAISGSGGSTYYADSVKGRFTISRDNSKNTLYLQMNSLRAEDTAVYYCARNYISMFDSWGQGTLVTVSSHHHHHHGAYPYDVPDYAS

SEQ ID NO: 54 - DNA, 777 bp, Homo sapiens
cagtctgtgctgactcagccaccctcagtgtcagtggccccaggaaagacggccaggattacctgtgggggaaacaacattggaagtaaaagtgtgcactggtaccagcagaggccaggccaggcccctgtgctggtcatctattatgatagcgaccggccctcagggatccctgagcgattctctggctccaactctgggaacacggccaccctgaccatcagcagggtcgaagccggggatgaggccgactattactgtcaggtgtgggatagtagtagtgattatgtcttcggaattgggaccaaggtcaccgtcctaggtggtggtggtggtagcggcggcggcggctctggtggtggtggatccgaggtgcagctggtggagtctggaggaggcttgatccagcctggggggtccctgagactctcctgtgcagcctctggattcacctttagcagctatgccatgagctgggtccgccaggctccagggaaggggctggagtgggtctcagctattagtggtagtggtggtagcacatactacgcagactccgtgaagggccggttcaccatctccagagacaattccaagaacacgctgtatctgcaaatgaacagcctgagagccgaggacacggccgtatattactgtgcgcgcaactacatctctatgttcgattcttggggtcaaggtactctggtgaccgtctcctcacaccatcaccatcaccatggcgcatacccgtacgacgttccggactacgcttcttag

SEQ ID NO: 55 - protein, 10 aa, Homo sapiens
QVWDSSSDHV

SEQ ID NO: 56 - protein, 10 aa, Homo sapiens
ARGYSSYYDA

SEQ ID NO: 57 - protein, 108 aa, Homo sapiens
QAVLTQPPSVSVAPGKTARITCGGNNIGSKSVHWYQQKPGQAPVLVIYYDSDRPSGIPERFSGSNSGNTATLTISRVEAGDEADYYCQVWDSSSDHVFGTGTKVTVLG

SEQ ID NO: 58 - DNA, 324 bp, Homo sapiens
caggctgtgctgactcagccaccctcagtgtcagtggccccaggaaagacggccaggattacctgtgggggaaacaacattggaagtaaaagtgtgcactggtaccagcagaagccaggccaggcccctgtgctggtcatctattatgatagcgaccggccctcagggatccctgagcgattctctggctccaactctgggaacacggccaccctgaccatcagcagggtcgaagccggggatgaggccgactattactgtcaggtgtgggatagtagtagtgatcatgtcttcggaactgggaccaaggtcaccgtcctaggt

SEQ ID NO: 59 - protein, 117 aa, Homo sapiens
QVQLVESGGGLVQPGGSLRLSCAASGFTFSSYAMSWVRQAPGKGLEWVSAISGSGGSTYYADSVKGRFTISRDNSKNTLYLQMNSLRAEDTAVYYCARGYSSYYDAWGQGTLVTVSS

SEQ ID NO: 60 - DNA, 351 bp, Homo sapiens
caggtgcagctggtggagtctgggggaggcttggtacagcctggggggtccctgagactctcctgtgcagcctctggattcacctttagcagctatgccatgagctgggtccgccaggctccagggaaggggctggagtgggtctcagctattagtggtagtggtggtagcacatactacgcagactccgtgaagggccggttcaccatctccagagacaattccaagaacacgctgtatctgcaaatgaacagcctgagagccgaggacacggccgtatattactgtgcgcgcggttactcttcttactacgatgcttggggtcaaggtactctggtgaccgtctcctca

SEQ ID NO: 61 - protein, 258 aa, Homo sapiens
QAVLTQPPSVSVAPGKTARITCGGNNIGSKSVHWYQQKPGQAPVLVIYYDSDRPSGIPERFSGSNSGNTATLTISRVEAGDEADYYCQVWDSSSDHVFGTGTKVTVLGGGGGSGGGGSGGGGSQVQLVESGGGLVQPGGSLRLSCAASGFTFSSYAMSWVRQAPGKGLEWVSAISGSGGSTYYADSVKGRFTISRDNSKNTLYLQMNSLRAEDTAVYYCARGYSSYYDAWGQGTLVTVSSHHHHHHGAYPYDVPDYAS

SEQ ID NO: 62 - DNA, 777 bp, Homo sapiens
caggctgtgctgactcagccaccctcagtgtcagtggccccaggaaagacggccaggattacctgtgggggaaacaacattggaagtaaaagtgtgcactggtaccagcagaagccaggccaggcccctgtgctggtcatctattatgatagcgaccggccctcagggatccctgagcgattctctggctccaactctgggaacacggccaccctgaccatcagcagggtcgaagccggggatgaggccgactattactgtcaggtgtgggatagtagtagtgatcatgtcttcggaactgggaccaaggtcaccgtcctaggtggtggtggtggtagcggcggcggcggctctggtggtggtggatcccaggtgcagctggtggagtctgggggaggcttggtacagcctggggggtccctgagactctcctgtgcagcctctggattcacctttagcagctatgccatgagctgggtccgccaggctccagggaaggggctggagtgggtctcagctattagtggtagtggtggtagcacatactacgcagactccgtgaagggccggttcaccatctccagagacaattccaagaacacgctgtatctgcaaatgaacagcctgagagccgaggacacggccgtatattactgtgcgcgcggttactcttcttactacgatgcttggggtcaaggtactctggtgaccgtctcctcacaccatcaccatcaccatggcgcatacccgtacgacgttccggactacgcttcttag

SEQ ID NO: 63 - protein, 8 aa, Homo sapiens
RSNIGENT

SEQ ID NO: 64 - protein, 11 aa, Homo sapiens
AAWDDRLNGYV

SEQ ID NO: 65 - protein, 8 aa, Homo sapiens
GYTFTNYG

SEQ ID NO: 66 - protein, 8 aa, Homo sapiens
IGAQKGDT

SEQ ID NO: 67 - protein, 10 aa, Homo sapiens
ARSQGVPFDS

SEQ ID NO: 68 - protein, 111 aa, Homo sapiens
QSVLTQPPSASGTPGQRVTISCSGSRSNIGENTVNWYQQLPGTAPKLLIYSNNQRPSGVPDRFSGSKSGTSASLAISGLHSDDEADYFCAAWDDRLNGYVFGTGTKVTVLG

SEQ ID NO: 69 - DNA, 333 bp, Homo sapiens
cagtctgtgttgactcagccaccctcagcgtctgggacccccgggcagagagtcaccatctcttgttctggaagcaggtccaacatcggagaaaatactgtcaactggtaccagcagctcccaggaacggcccccaaactcctcatctacagtaataatcagcggccctcaggggtccctgaccgattctctggctccaagtctggcacctcagcctccctggccatcagtgggcttcactctgacgatgaggctgactatttttgtgcagcatgggatgaccgcctcaatggttatgtcttcggaactgggaccaaggtcaccgtcctaggt

SEQ ID NO: 70 - protein, 117 aa, Homo sapiens
QVQLVQSGPEVKKPGASVKVSCKASGYTFTNYGFTWVRQAPGQGLEWMGWIGAQKGDTEYAQKFQGRVTMTTDTSTSTVYLELRSLRSDDTAVYYCARSQGVPFDSWGQGTLVTVSS

SEQ ID NO: 71 - DNA, 351 bp, Homo sapiens
caggtgcagctggtgcaatctggacctgaggtgaagaagcctggggcctcggtgaaggtctcctgcaaggcttctggttacacctttaccaactatggtttcacctgggtgcgacaggcccctggacaaggtcttgagtggatgggatggatcggcgctcaaaagggtgacacagagtatgcacaaaaattccagggcagagtcaccatgacgacagacacatccacgagcacagtctacttggagttgaggagcctgaggtctgacgacacggccgtgtattactgtgcgcgctctcagggtgttccgttcgattcttggggtcaaggtactctggtgaccgtctcctca

SEQ ID NO: 72 - protein, 261 aa, Homo sapiens
QSVLTQPPSASGTPGQRVTISCSGSRSNIGENTVNWYQQLPGTAPKLLIYSNNQRPSGVPDRFSGSKSGTSASLAISGLHSDDEADYFCAAWDDRLNGYVFGTGTKVTVLGGGGGSGGGGSGGGGSQVQLVQSGPEVKKPGASVKVSCKASGYTFTNYGFTWVRQAPGQGLEWMGWIGAQKGDTEYAQKFQGRVTMTTDTSTSTVYLELRSLRSDDTAVYYCARSQGVPFDSWGQGTLVTVSSHHHHHHGAYPYDVPDYAS

SEQ ID NO: 73 - DNA, 786 bp, Homo sapiens
cagtctgtgttgactcagccaccctcagcgtctgggacccccgggcagagagtcaccatctcttgttctggaagcaggtccaacatcggagaaaatactgtcaactggtaccagcagctcccaggaacggcccccaaactcctcatctacagtaataatcagcggccctcaggggtccctgaccgattctctggctccaagtctggcacctcagcctccctggccatcagtgggcttcactctgacgatgaggctgactatttttgtgcagcatgggatgaccgcctcaatggttatgtcttcggaactgggaccaaggtcaccgtcctaggtggtggtggtggtagcggcggcggcggctctggtggtggtggatcccaggtgcagctggtgcaatctggacctgaggtgaagaagcctggggcctcggtgaaggtctcctgcaaggcttctggttacacctttaccaactatggtttcacctgggtgcgacaggcccctggacaaggtcttgagtggatgggatggatcggcgctcaaaagggtgacacagagtatgcacaaaaattccagggcagagtcaccatgacgacagacacatccacgagcacagtctacttggagttgaggagcctgaggtctgacgacacggccgtgtattactgtgcgcgctctcagggtgttccgttcgattcttggggtcaaggtactctggtgaccgtctcctcacaccatcaccatcaccatggcgcatacccgtacgacgttccggactacgcttcttag

SEQ ID NO: 74 - protein, 8 aa, Homo sapiens
RSNIGSNT

SEQ ID NO: 75 - protein, 11 aa, Homo sapiens
ATWDDSLNEYV

SEQ ID NO: 76 - protein, 8 aa, Homo sapiens
GYTFTRYG

SEQ ID NO: 77 - protein, 8 aa, Homo sapiens
ISGYNGNT

SEQ ID NO: 78 - protein, 10 aa, Homo sapiens
ARHGYGYHGD

SEQ ID NO: 79 - protein, 111 aa, Homo sapiens
QSVLTQPPSASATPGQRGTISCSGGRSNIGSNTVNWYQQLPGTAPKLLIYNNNLRPSGVPDRFSGSKSGTSASLAIRGLQSEDEADYYCATWDDSLNEYVFGTGTKVTVLG

SEQ ID NO: 80 - DNA, 333 bp, Homo sapiens
cagtctgtgttgactcagccaccctcagcgtctgcgacccccgggcagaggggcaccatttcgtgttctggaggcaggtccaacatcggaagtaacactgttaactggtaccagcagctcccaggaacggcccccaaactcctcatctataataataatctgcggccctcaggggtccctgaccgattctctggctccaagtctggcacctcagcctccctggccatcagggggctccagtctgaggatgaggctgattattactgtgcaacatgggatgacagcctgaatgaatatgtcttcggaactgggaccaaggtcaccgtcctaggt

SEQ ID NO: 81 - protein, 117 aa, Homo sapiens
QVQLVQSGAEVKKPGASVKVSCKASGYTFTRYGISWVRQAPGQGLEWMGWISGYNGNTNYAQKLQGRVTMTTDTSTSTAYMELRSLRSDDTAVYYCARHGYGYHGDWGQGTLVTVSS

SEQ ID NO: 82 - DNA, 351 bp, Homo sapiens
caggtgcagctggtgcaatctggagctgaggtgaagaagcctggggcctcagtgaaggtctcctgcaaggcttctggttacacctttaccagatatggtatcagctgggtgcgacaggcccctggacaagggcttgagtggatgggatggatcagcggttacaacggtaacacaaactatgcacagaagctccagggcagagtcaccatgaccacagacacatccacgagcacagcctacatggagctgaggagcctgaggtctgacgacacggccgtgtattactgtgcgcgccatggttacggttaccatggtgattggggtcaaggtactctggtgaccgtctcctca

SEQ ID NO: 83 - protein, 261 aa, Homo sapiens
QSVLTQPPSASATPGQRGTISCSGGRSNIGSNTVNWYQQLPGTAPKLLIYNNNLRPSGVPDRFSGSKSGTSASLAIRGLQSEDEADYYCATWDDSLNEYVFGTGTKVTVLGGGGGSGGGGSGGGGSQVQLVQSGAEVKKPGASVKVSCKASGYTFTRYGISWVRQAPGQGLEWMGWISGYNGNTNYAQKLQGRVTMTTDTSTSTAYMELRSLRSDDTAVYYCARHGYGYHGDWGQGTLVTVSSHHHHHHGAYPYDVPDYAS

SEQ ID NO: 84 - DNA, 786 bp, Homo sapiens
cagtctgtgttgactcagccaccctcagcgtctgcgacccccgggcagaggggcaccatttcgtgttctggaggcaggtccaacatcggaagtaacactgttaactggtaccagcagctcccaggaacggcccccaaactcctcatctataataataatctgcggccctcaggggtccctgaccgattctctggctccaagtctggcacctcagcctccctggccatcagggggctccagtctgaggatgaggctgattattactgtgcaacatgggatgacagcctgaatgaatatgtcttcggaactgggaccaaggtcaccgtcctaggtggtggtggtggtagcggcggcggcggctctggtggtggtggatcccaggtgcagctggtgcaatctggagctgaggtgaagaagcctggggcctcagtgaaggtctcctgcaaggcttctggttacacctttaccagatatggtatcagctgggtgcgacaggcccctggacaagggcttgagtggatgggatggatcagcggttacaacggtaacacaaactatgcacagaagctccagggcagagtcaccatgaccacagacacatccacgagcacagcctacatggagctgaggagcctgaggtctgacgacacggccgtgtattactgtgcgcgccatggttacggttaccatggtgattggggtcaaggtactctggtgaccgtctcctcacaccatcaccatcaccatggcgcatacccgtacgacgttccggactacgcttcttag

SEQ ID NO: 85 - protein, 9 aa, Homo sapiens
SSNIGAGYV

SEQ ID NO: 86 - protein, 11 aa, Homo sapiens
QSYDSSLSGWV

SEQ ID NO: 87 - protein, 8 aa, Homo sapiens
GFTFKDYY

SEQ ID NO: 88 - protein, 8 aa, Homo sapiens
ISTSGNSV

SEQ ID NO: 89 - protein, 11 aa, Homo sapiens
ARSPGHSDYDS

SEQ ID NO: 90 - protein, 112 aa, Homo sapiens
QSVLTQPPSVSGAPGQRVTISCTGSSSNIGAGYVVQWYQQLPGTAPKLLIYHNNDRPSGVPYRFSGSKSGTSASLAITGLQAEDEADYYCQSYDSSLSGWVFGGGTKLTVLG

SEQ ID NO: 91 - DNA, 336 bp, Homo sapiens
cagtctgtgctgacgcagccgccctcagtgtctggggccccagggcagagggtcaccatctcctgtactgggagcagctccaacatcggggcaggttatgttgtacagtggtatcagcagcttccaggaacagcccccaaactcctcatctatcataacaacgatcggccctcaggggtcccttaccgattctctggctccaagtctggcacctcagcctccctggccatcactgggctccaggctgaggatgaggctgattattactgccagtcctatgacagcagcctgagtggttgggtgttcggcggagggaccaagctgaccgtcctaggt

SEQ ID NO: 92 - protein, 118 aa, Homo sapiens
EVQLVESGGGLVKPGGSLRLSCAASGFTFKDYYMNWIRQAPGKGLEWISHISTSGNSVDYADSVKGRFTISRDNAKNSLYLQMNSLRAEDTAVYYCARSPGHSDYDSWGQGTLVTVSS

SEQ ID NO: 93 - DNA, 354 bp, Homo sapiens
gaggtgcagctggtggagtctgggggaggcctagtcaagcctggagggtccctgagactctcctgtgcagcctctggattcacctttaaagactactacatgaactggatccgccaggctccagggaagggcctggagtggatttcacacattagtaccagcggtaatagtgtagattatgcagactctgtcaagggccggttcaccatctccagggacaacgccaagaattcactgtacctgcaaatgaacagcctgagagccgaggacacggccgtatattactgtgcgcgctctccgggtcattctgactacgattcttggggtcaaggtactctggtgaccgtctcctca

SEQ ID NO: 94 - protein, 263 aa, Homo sapiens
QSVLTQPPSVSGAPGQRVTISCTGSSSNIGAGYVVQWYQQLPGTAPKLLIYHNNDRPSGVPYRFSGSKSGTSASLAITGLQAEDEADYYCQSYDSSLSGWVFGGGTKLTVLGGGGGSGGGGSGGGGSEVQLVESGGGLVKPGGSLRLSCAASGFTFKDYYMNWIRQAPGKGLEWISHISTSGNSVDYADSVKGRFTISRDNAKNSLYLQMNSLRAEDTAVYYCARSPGHSDYDSWGQGTLVTVSSHHHHHHGAYPYDVPDYAS

SEQ ID NO: 95 - DNA, 792 bp, Homo sapiens
cagtctgtgctgacgcagccgccctcagtgtctggggccccagggcagagggtcaccatctcctgtactgggagcagctccaacatcggggcaggttatgttgtacagtggtatcagcagcttccaggaacagcccccaaactcctcatctatcataacaacgatcggccctcaggggtcccttaccgattctctggctccaagtctggcacctcagcctccctggccatcactgggctccaggctgaggatgaggctgattattactgccagtcctatgacagcagcctgagtggttgggtgttcggcggagggaccaagctgaccgtcctaggtggtggtggtggtagcggcggcggcggctctggtggtggtggatccgaggtgcagctggtggagtctgggggaggcctagtcaagcctggagggtccctgagactctcctgtgcagcctctggattcacctttaaagactactacatgaactggatccgccaggctccagggaagggcctggagtggatttcacacattagtaccagcggtaatagtgtagattatgcagactctgtcaagggccggttcaccatctccagggacaacgccaagaattcactgtacctgcaaatgaacagcctgagagccgaggacacggccgtatattactgtgcgcgctctccgggtcattctgactacgattcttggggtcaaggtactctggtgaccgtctcctcacaccatcaccatcaccatggcgcatacccgtacgacgttccggactacgcttcttag

SEQ ID NO: 96 - protein, 6 aa, Homo sapiens
NIGDKS

SEQ ID NO: 97 - protein, 13 aa, Homo sapiens
QVWASGTDHPYVI

SEQ ID NO: 98 - protein, 10 aa, Homo sapiens
ARMYGSYTDM

SEQ ID NO: 99 - protein, 111 aa, Homo sapiens
SYVLTQPPSVSVAPGKTARITCGGNNIGDKSVHWYQQKPGQAPVLVIYYDSDRPSGIPERFSGSNSGNTATLTISRVEAGDEADYYCQVWASGTDHPYVIFGGGTKVTVLG

SEQ ID NO: 100 - DNA, 333 bp, Homo sapiens
tcctatgtgctgactcagccaccctcagtgtcagtggccccaggaaagacggccaggattacctgtgggggaaacaacattggagataaaagtgtgcactggtaccagcagaagccaggccaggcccctgtgctggtcatctattatgatagcgaccggccctcagggatccctgagcgattctctggctccaactctgggaacacggccaccctgaccatcagcagggtcgaagccggggacgaggccgactattactgtcaggtgtgggctagtggtactgatcatccctatgtgatattcggcggagggaccaaggtcaccgtcctaggt

SEQ ID NO: 101 - protein, 117 aa, Homo sapiens
EVQLVESGGGLVQPGGSLRLSCAASGFTFSSYAMSWVRQAPGKGLEWVSAISGSGGSTYYADSVKGRFTISRDNSKNTLYLQMNSLRAEDTAVYYCARMYGSYTDMWGQGTLVTVSS

SEQ ID NO: 102 - DNA, 351 bp, Homo sapiens
gaggtgcagctggtggagtctgggggaggcttggtacagcctggggggtccctgagactctcctgtgcagcctctggattcacctttagcagctatgccatgagctgggtccgccaggctccagggaaggggctggagtgggtctcagctattagtggtagtggtggtagcacatactacgcagactccgtgaagggccggttcaccatctccagagacaattccaagaacacgctgtatctgcaaatgaacagcctgagagccgaggacacggccgtatattactgtgcgcgcatgtacggttcttacactgatatgtggggtcaaggtactctggtgaccgtctcctca

SEQ ID NO: 103 - protein, 261 aa, Homo sapiens
SYVLTQPPSVSVAPGKTARITCGGNNIGDKSVHWYQQKPGQAPVLVIYYDSDRPSGIPERFSGSNSGNTATLTISRVEAGDEADYYCQVWASGTDHPYVIFGGGTKVTVLGGGGGSGGGGSGGGGSEVQLVESGGGLVQPGGSLRLSCAASGFTFSSYAMSWVRQAPGKGLEWVSAISGSGGSTYYADSVKGRFTISRDNSKNTLYLQMNSLRAEDTAVYYCARMYGSYTDMWGQGTLVTVSSHHHHHHGAYPYDVPDYAS

SEQ ID NO: 104 - DNA, 786 bp, Homo sapiens
tcctatgtgctgactcagccaccctcagtgtcagtggccccaggaaagacggccaggattacctgtgggggaaacaacattggagataaaagtgtgcactggtaccagcagaagccaggccaggcccctgtgctggtcatctattatgatagcgaccggccctcagggatccctgagcgattctctggctccaactctgggaacacggccaccctgaccatcagcagggtcgaagccggggacgaggccgactattactgtcaggtgtgggctagtggtactgatcatccctatgtgatattcggcggagggaccaaggtcaccgtcctaggtggtggtggtggtagcggcggcggcggctctggtggtggtggatccgaggtgcagctggtggagtctgggggaggcttggtacagcctggggggtccctgagactctcctgtgcagcctctggattcacctttagcagctatgccatgagctgggtccgccaggctccagggaaggggctggagtgggtctcagctattagtggtagtggtggtagcacatactacgcagactccgtgaagggccggttcaccatctccagagacaattccaagaacacgctgtatctgcaaatgaacagcctgagagccgaggacacggccgtatattactgtgcgcgcatgtacggttcttacactgatatgtggggtcaaggtactctggtgaccgtctcctcacaccatcaccatcaccatggcgcatacccgtacgacgttccggactacgcttcttag

SEQ ID NO: 105 - protein, 8 aa, Homo sapiens
SSNIGYNY

SEQ ID NO: 106 - protein, 11 aa, Homo sapiens
TSWDDSLSGYV

SEQ ID NO: 107 - protein, 8 aa, Homo sapiens
GNAFTNFY

SEQ ID NO: 108 - protein, 9 aa, Homo sapiens
INPSGTDLT

SEQ ID NO: 109 - protein, 13 aa, Homo sapiens
ARQYAYGYSGFDM

SEQ ID NO: 110 - protein, 111 aa, Homo sapiens
QSVLTQPPSASGTPGQRVTISCSGSSSNIGYNYVYWYQQLPGTAPKLLISRNNQRPSGVPDRFSGSKSGTSASLAISGLRSEDEADYYCTSWDDSLSGYVFGPGTKVTVLG

SEQ ID NO: 111 - DNA, 333 bp, Homo sapiens
cagtctgtgctgactcagccaccctcagcgtctgggacccccgggcagagggtcaccatctcttgttctggaagcagctccaacatcggatataattatgtatactggtaccagcagctcccaggaacggcccccaaactcctcatctctagaaataatcagcggccctcaggggtccctgaccgattctctggctccaagtctggcacctcagcctccctggccatcagtgggctccggtccgaggatgaggctgactattactgtacatcgtgggatgacagcctgagtggttatgtcttcggacctgggaccaaggtcaccgtcctaggt

SEQ ID NO: 112 - protein, 121 aa, Homo sapiens
EVQLVQSGAEVKKPGASVKVSCKASGNAFTNFYIHWVRQAPGQGLEWMGLINPSGTDLTRYAQKFQGRVTMTRDTPTSTVYMELSSLRSDDTAVYYCARQYAYGYSGFDMWGQGTLVTVSS

SEQ ID NO: 113 - DNA, 363 bp, Homo sapiens
gaagtgcagctggtgcagtctggggctgaggtgaagaagcctggggcctcagtgaaggtttcctgcaaggcatctggaaacgccttcaccaacttctatatacactgggtgcgacaggcccctggacaagggcttgagtggatgggattaatcaaccctagtggtactgacctcacaaggtacgcacagaagttccagggcagagtcaccatgaccagggacacgcccacgagcacagtctacatggagctgagcagcctgaggtctgacgacacggctgtgtattactgtgcgcgccagtacgcttacggttactctggtttcgatatgtggggtcaaggtactctggtgaccgtctcctca

SEQ ID NO: 114 - protein, 265 aa, Homo sapiens
QSVLTQPPSASGTPGQRVTISCSGSSSNIGYNYVYWYQQLPGTAPKLLISRNNQRPSGVPDRFSGSKSGTSASLAISGLRSEDEADYYCTSWDDSLSGYVFGPGTKVTVLGGGGGSGGGGSGGGGSEVQLVQSGAEVKKPGASVKVSCKASGNAFTNFYIHWVRQAPGQGLEWMGLINPSGTDLTRYAQKFQGRVTMTRDTPTSTVYMELSSLRSDDTAVYYCARQYAYGYSGFDMWGQGTLVTVSSHHHHHHGAYPYDVPDYAS

SEQ ID NO: 115 - DNA, 798 bp, Homo sapiens
cagtctgtgctgactcagccaccctcagcgtctgggacccccgggcagagggtcaccatctcttgttctggaagcagctccaacatcggatataattatgtatactggtaccagcagctcccaggaacggcccccaaactcctcatctctagaaataatcagcggccctcaggggtccctgaccgattctctggctccaagtctggcacctcagcctccctggccatcagtgggctccggtccgaggatgaggctgactattactgtacatcgtgggatgacagcctgagtggttatgtcttcggacctgggaccaaggtcaccgtcctaggtggtggtggtggtagcggcggcggcggctctggtggtggtggatccgaagtgcagctggtgcagtctggggctgaggtgaagaagcctggggcctcagtgaaggtttcctgcaaggcatctggaaacgccttcaccaacttctatatacactgggtgcgacaggcccctggacaagggcttgagtggatgggattaatcaaccctagtggtactgacctcacaaggtacgcacagaagttccagggcagagtcaccatgaccagggacacgcccacgagcacagtctacatggagctgagcagcctgaggtctgacgacacggctgtgtattactgtgcgcgccagtacgcttacggttactctggtttcgatatgtggggtcaaggtactctggtgaccgtctcctcacaccatcaccatcaccatggcgcatacccgtacgacgttccggactacgcttcttag

SEQ ID NO: 116 - protein, 6 aa, Homo sapiens
QSVSNW

SEQ ID NO: 117 - protein, 9 aa, Homo sapiens
QQSYSTPIT

SEQ ID NO: 118 - protein, 8 aa, Homo sapiens
GYTFTSYY

SEQ ID NO: 119 - protein, 8 aa, Homo sapiens
INPNTGGS

SEQ ID NO: 120 - protein, 9 aa, Homo sapiens
ARGDVTYDE

SEQ ID NO: 121 - protein, 108 aa, Homo sapiens
DIQMTQSPSSVSASVGDRVTITCRASQSVSNWLAWYQLKPGKAPKLLIYAASSLQSGVPSRFSGSGSGTDFTLTISSLQPEDFATYYCQQSYSTPITFGGGTKVEIKR

SEQ ID NO: 122 - DNA, 324 bp, Homo sapiens
gacatccagatgacccagtctccatcttccgtgtctgcatctgtaggagacagagtcaccatcacttgtcgggcgagtcagagtgttagcaactggttagcctggtatcaactgaaaccagggaaagcccctaagctcctgatctatgctgcatccagtttgcaaagtggggtcccatcaaggttcagtggcagtggatctgggacagatttcactctcaccatcagcagtctgcaacctgaagattttgcaacttactactgtcaacagagttacagtaccccgatcaccttcggcggagggaccaaggtggagatcaaacgt

SEQ ID NO: 123 - protein, 116 aa, Homo sapiens
QVQLVQSGAEVKKPGTSVKVSCKASGYTFTSYYIHWVRQAPGQGLEWMGWINPNTGGSNFAQKFQGRVTMTRDTSISTAYMELNRLRSDDTAVYYCARGDVTYDEWGQGTLVTVSS

SEQ ID NO: 124 - DNA, 348 bp, Homo sapiens
caggtccagctggtacagtctggggctgaggtgaagaagcctgggacctcagtgaaggtctcctgcaaggcttctggatacaccttcacctcctactatatacactgggtgcgacaggcccctggacaagggcttgagtggatgggatggatcaaccctaacactggtggctcaaactttgcacagaagtttcagggcagggtcaccatgaccagggacacgtccatcagcacagcctacatggagctgaacaggctgaggtctgacgacacggccgtgtattactgtgcgcgcggtgacgttacttacgatgaatggggtcaaggtactctggtgaccgtctcctca

SEQ ID NO: 125 - protein, 257 aa, Homo sapiens
DIQMTQSPSSVSASVGDRVTITCRASQSVSNWLAWYQLKPGKAPKLLIYAASSLQSGVPSRFSGSGSGTDFTLTISSLQPEDFATYYCQQSYSTPITFGGGTKVEIKRGGGGSGGGGSGGGGSQVQLVQSGAEVKKPGTSVKVSCKASGYTFTSYYIHWVRQAPGQGLEWMGWINPNTGGSNFAQKFQGRVTMTRDTSISTAYMELNRLRSDDTAVYYCARGDVTYDEWGQGTLVTVSSHHHHHHGAYPYDVPDYAS

SEQ ID NO: 126 - DNA, 774 bp, Homo sapiens
gacatccagatgacccagtctccatcttccgtgtctgcatctgtaggagacagagtcaccatcacttgtcgggcgagtcagagtgttagcaactggttagcctggtatcaactgaaaccagggaaagcccctaagctcctgatctatgctgcatccagtttgcaaagtggggtcccatcaaggttcagtggcagtggatctgggacagatttcactctcaccatcagcagtctgcaacctgaagattttgcaacttactactgtcaacagagttacagtaccccgatcaccttcggcggagggaccaaggtggagatcaaacgtggtggtggtggtagcggcggcggcggctctggtggtggtggatcccaggtccagctggtacagtctggggctgaggtgaagaagcctgggacctcagtgaaggtctcctgcaaggcttctggatacaccttcacctcctactatatacactgggtgcgacaggcccctggacaagggcttgagtggatgggatggatcaaccctaacactggtggctcaaactttgcacagaagtttcagggcagggtcaccatgaccagggacacgtccatcagcacagcctacatggagctgaacaggctgaggtctgacgacacggccgtgtattactgtgcgcgcggtgacgttacttacgatgaatggggtcaaggtactctggtgaccgtctcctcacaccatcaccatcaccatggcgcatacccgtacgacgttccggactacgcttcttag

SEQ ID NO: 127 - protein, 10 aa, Homo sapiens
QVWDINDHYV

SEQ ID NO: 128 - protein, 10 aa, Homo sapiens
ARSQASFMDI

SEQ ID NO: 129 - protein, 108 aa, Homo sapiens
SYELTQPPSVSVAPGKTASITCGGNNIGSKSVHWYQQKPGQAPVLVIYYDDMRPSGIPERFSGSSSGNTATLTISPVEAGDEADYYCQVWDINDHYVFASGTKVTVLG

SEQ ID NO: 130 - DNA, 324 bp, Homo sapiens
tcctatgagctgactcagccaccctcagtgtcagtggccccaggaaagacggccagcattacctgtgggggaaacaacattggaagtaaaagtgtgcactggtaccagcagaagccaggccaggcccctgtgctggtcatctattatgatgacatgcggccctcaggtatccctgagcgattctctggctccagctctgggaacacggccaccctgaccatcagcccggtcgaagccggggatgaggccgactattactgtcaggtgtgggatattaatgatcattatgtcttcgcatcggggaccaaggtcaccgtcctaggt

SEQ ID NO: 131 - protein, 117 aa, Homo sapiens
EVQLVESGGGLVQPGGSLRLSCAASGFTFSSYAMSWVRQAPGKGLEWVSAISGSGGSTYYADSVKGRFTISRDNSKNTLYLQMNSLRAEDTAVYYCARSQASFMDIWGQGTLVTVSS

SEQ ID NO: 132 - DNA, 351 bp, Homo sapiens
gaggtgcagctggtggagtctgggggaggcttggtacagcctggggggtccctgagactctcctgtgcagcctctggattcacctttagcagctatgccatgagctgggtccgccaggctccagggaaggggctggagtgggtctcagctattagtggtagtggtggtagcacatactacgcagactccgtgaagggccggttcaccatctccagagacaattccaagaacacgctgtatctgcaaatgaacagcctgagagccgaggacacggccgtatattactgtgcgcgctctcaggcttctttcatggatatctggggtcaaggtactctggtgaccgtctcctca

SEQ ID NO: 133 - protein, 258 aa, Homo sapiens
SYELTQPPSVSVAPGKTASITCGGNNIGSKSVHWYQQKPGQAPVLVIYYDDMRPSGIPERFSGSSSGNTATLTISPVEAGDEADYYCQVWDINDHYVFASGTKVTVLGGGGGSGGGGSGGGGSEVQLVESGGGLVQPGGSLRLSCAASGFTFSSYAMSWVRQAPGKGLEWVSAISGSGGSTYYADSVKGRFTISRDNSKNTLYLQMNSLRAEDTAVYYCARSQASFMDIWGQGTLVTVSSHHHHHHGAYPYDVPDYAS

SEQ ID NO: 134 - DNA, 777 bp, Homo sapiens
tcctatgagctgactcagccaccctcagtgtcagtggccccaggaaagacggccagcattacctgtgggggaaacaacattggaagtaaaagtgtgcactggtaccagcagaagccaggccaggcccctgtgctggtcatctattatgatgacatgcggccctcaggtatccctgagcgattctctggctccagctctgggaacacggccaccctgaccatcagcccggtcgaagccggggatgaggccgactattactgtcaggtgtgggatattaatgatcattatgtcttcgcatcggggaccaaggtcaccgtcctaggtggtggtggtggtagcggcggcggcggctctggtggtggtggatccgaggtgcagctggtggagtctgggggaggcttggtacagcctggggggtccctgagactctcctgtgcagcctctggattcacctttagcagctatgccatgagctgggtccgccaggctccagggaaggggctggagtgggtctcagctattagtggtagtggtggtagcacatactacgcagactccgtgaagggccggttcaccatctccagagacaattccaagaacacgctgtatctgcaaatgaacagcctgagagccgaggacacggccgtatattactgtgcgcgctctcaggcttctttcatggatatctggggtcaaggtactctggtgaccgtctcctcacaccatcaccatcaccatggcgcatacccgtacgacgttccggactacgcttcttag

SEQ ID NO: 135 - protein, 11 aa, Homo sapiens
QVWDSSSDQGV

SEQ ID NO: 136 - protein, 7 aa, Homo sapiens
IGTGGGT

SEQ ID NO: 137 - protein, 10 aa, Homo sapiens
ARGTGYDGDQ

SEQ ID NO: 138 - protein, 109 aa, Homo sapiens
LPVLTQPPSVSVAPGQTARITCGGNNIGSKSVHWYQQKPGQAPVLVVYDDSDRPSGIPERFSGSNSGNTATLTISRVEAGDEADYYCQVWDSSSDQGVFGTGTKVTVLG

SEQ ID NO: 139 - DNA, 327 bp, Homo sapiens
ctgcctgtgctgactcagccaccctcggtgtcagtggccccaggacagacggccaggatcacctgtgggggaaacaacattggaagtaaaagtgtgcactggtaccagcagaagccaggccaggcccctgtgctggtcgtctatgatgatagcgaccggccctcagggatccctgagcgattctctggctccaattctgggaacacggccaccctgaccatcagcagggtcgaagccggggatgaggccgactattactgtcaggtgtgggatagtagtagtgatcagggcgtcttcggaactgggaccaaggtcaccgtcctaggt

SEQ ID NO: 140 - protein, 116 aa, Homo sapiens
EVQLVQSGGGLVQPRGSLRLSCAGSGFTFSSYAMHWVRQAPGKGLEWVSAIGTGGGTYYADSVKGRFTISRDNAKNSLYLQMNSLRAEDTAMYYCARGTGYDGDQWGQGTLVTVSS

SEQ ID NO: 141 - DNA, 348 bp, Homo sapiens
gaagtgcagctggtgcagtctgggggaggcttggtacagcctagggggtccctgagactctcctgtgcaggctctggattcaccttcagtagctatgctatgcactgggttcgccaggctccaggaaaaggtctggagtgggtatcagctattggtactggtggtggcacatactatgcagactccgtgaagggccgattcaccatctccagggacaatgccaagaactccttgtatcttcaaatgaacagcctgagagccgaggacaccgccatgtattactgtgcgcgcggtactggttacgacggtgatcagtggggtcaaggtactctggtgaccgtctcctca

SEQ ID NO: 142 - protein, 258 aa, Homo sapiens
LPVLTQPPSVSVAPGQTARITCGGNNIGSKSVHWYQQKPGQAPVLVVYDDSDRPSGIPERFSGSNSGNTATLTISRVEAGDEADYYCQVWDSSSDQGVFGTGTKVTVLGGGGGSGGGGSGGGGSEVQLVQSGGGLVQPRGSLRLSCAGSGFTFSSYAMHWVRQAPGKGLEWVSAIGTGGGTYYADSVKGRFTISRDNAKNSLYLQMNSLRAEDTAMYYCARGTGYDGDQWGQGTLVTVSSHHHHHHGAYPYDVPDYAS

SEQ ID NO: 143 - DNA, 777 bp, Homo sapiens
ctgcctgtgctgactcagccaccctcggtgtcagtggccccaggacagacggccaggatcacctgtgggggaaacaacattggaagtaaaagtgtgcactggtaccagcagaagccaggccaggcccctgtgctggtcgtctatgatgatagcgaccggccctcagggatccctgagcgattctctggctccaattctgggaacacggccaccctgaccatcagcagggtcgaagccggggatgaggccgactattactgtcaggtgtgggatagtagtagtgatcagggcgtcttcggaactgggaccaaggtcaccgtcctaggtggtggtggtggtagcggcggcggcggctctggtggtggtggatccgaagtgcagctggtgcagtctgggggaggcttggtacagcctagggggtccctgagactctcctgtgcaggctctggattcaccttcagtagctatgctatgcactgggttcgccaggctccaggaaaaggtctggagtgggtatcagctattggtactggtggtggcacatactatgcagactccgtgaagggccgattcaccatctccagggacaatgccaagaactccttgtatcttcaaatgaacagcctgagagccgaggacaccgccatgtattactgtgcgcgcggtactggttacgacggtgatcagtggggtcaaggtactctggtgaccgtctcctcacaccatcaccatcaccatggcgcatacccgtacgacgttccggactacgcttcttag